European Patent Application EP 4 537 841 A1, published April 16, 2025. Title: A pharmaceutical composition comprising an anti-integrin alpha 11 antibody for the treatment or prevention of age-related diseases. Applicant: Astellas Pharma Inc. The sequence listing filed with the application follows.

SEQUENCE LISTING (4 sequences)

SEQ ID NO: 1 - DNA, 1350 bp, synthetic construct
  misc_feature 1..1350: note = DNA encoding heavy-chain of #014
  source 1..1350: mol_type = other DNA
gaggtgcagttggttgaatctggcggcggattggttcagcctggcggatctctgagactgtcttgtgccgcctctggcttcaacctgacctcctcctacatccactgggtccgacaggcccctggcaaaggattggaatgggtcgcctctatctccagccactccagctacacctactacgccgactccgtgaagggcagattcaccatctctgccgacacctccaagaacaccgcctacctgcagatgaactccctgagagccgaggacaccgccgtgtactactgtgccagatactggtactactccgcctgggctctcgactattggggccagggaacactggtcaccgtgtcctctgctaagaccaccgctcctagcgtgtaccctctggctcctgtgtgtggcgataccaccggatcctctgtgaccctgggatgtctggtcaagggctacttccccgagcctgtgacactgacctggaactctggatctctgtcctctggcgtgcacacctttccagccgtgctgcagtctgacctgtacaccctgtcctcttccgtgaccgtgacatcctccacctggcctagccagtccatcacctgtaacgtggcccatcctgcctccagcaccaaggtggacaagaagatcgagcctcggggccctaccatcaagccttgtcctccatgcaagtgccccgctcctaatctgctcggaggcccttccgtgttcatcttcccacctaagatcaaggacgtgctgatgatctccctgtctcctatcgtgacctgcgtggtggtggacgtgtccgaggatgatcctgacgtgcagatcagttggttcgtgaacaacgtggaagtgcacaccgctcagacccagacacacagagaggactacaacagcaccctgagagtggtgtctgccctgcctatccagcatcaggattggatgtccggcaaagagttcaagtgcaaagtgaacaacaaggacctgcctgctccaatcgagcggaccatctctaagcctaagggctctgtcagggcccctcaggtgtacgttttgccacctcctgaggaagagatgaccaagaaacaagtgaccctgacatgcatggtcaccgacttcatgcccgaggacatctacgtggaatggaccaacaacggcaagaccgagctgaactacaagaataccgagccagtgctggactccgacggctcctacttcatgtactccaagctgcgcgtcgagaagaagaactgggtcgagagaaactcctactcctgctccgtggtgcacgagggcctgcacaatcaccacaccaccaagtccttctctcggacccctggaaaa

SEQ ID NO: 2 - protein, 450 aa, synthetic construct
  REGION 1..450: note = heavy-chain of #014
EVQLVESGGGLVQPGGSLRLSCAASGFNLTSSYIHWVRQAPGKGLEWVASISSHSSYTYYADSVKGRFTISADTSKNTAYLQMNSLRAEDTAVYYCARYWYYSAWALDYWGQGTLVTVSSAKTTAPSVYPLAPVCGDTTGSSVTLGCLVKGYFPEPVTLTWNSGSLSSGVHTFPAVLQSDLYTLSSSVTVTSSTWPSQSITCNVAHPASSTKVDKKIEPRGPTIKPCPPCKCPAPNLLGGPSVFIFPPKIKDVLMISLSPIVTCVVVDVSEDDPDVQISWFVNNVEVHTAQTQTHREDYNSTLRVVSALPIQHQDWMSGKEFKCKVNNKDLPAPIERTISKPKGSVRAPQVYVLPPPEEEMTKKQVTLTCMVTDFMPEDIYVEWTNNGKTELNYKNTEPVLDSDGSYFMYSKLRVEKKNWVERNSYSCSVVHEGLHNHHTTKSFSRTPGK

SEQ ID NO: 3 - DNA, 648 bp, synthetic construct
  misc_feature 1..648: note = DNA encoding light-chain of #014
  source 1..648: mol_type = other DNA
gacatccagatgacccagtctccatcctctctgtccgcctctgtgggcgacagagtgaccatcacctgtcgggcttctcagtccgtgtctagcgccgtggcttggtatcagcagaagcctggcaaggcccctaagctgctgatctactccgcctccagcctgtactctggcgtgccctctagattctccggctctagatctggcaccgactttaccctgacaatcagctccctgcagcctgaggacttcgccacctactactgccagcagagcgccccttactcctctctgatcacctttggccagggcaccaaggtggaaatcaagagagctgacgccgctcctaccgtgtctatcttcccacctagctccgagcagctgacctctggcggagcttctgtcgtgtgcttcctgaacaacttctaccccaaggacatcaacgtgaagtggaagatcgacggctccgagagacagaacggcgtgctgaactcttggaccgaccaggactccaaggacagcacctactccatgtcctccacactgaccctgaccaaggacgagtacgagcggcacaactcctatacctgcgaggctacccacaagacctccacctctccaatcgtgaagtccttcaaccggaacgagtgc

SEQ ID NO: 4 - protein, 216 aa, synthetic construct
  REGION 1..216: note = light-chain of #014
DIQMTQSPSSLSASVGDRVTITCRASQSVSSAVAWYQQKPGKAPKLLIYSASSLYSGVPSRFSGSRSGTDFTLTISSLQPEDFATYYCQQSAPYSSLITFGQGTKVEIKRADAAPTVSIFPPSSEQLTSGGASVVCFLNNFYPKDINVKWKIDGSERQNGVLNSWTDQDSKDSTYSMSSTLTLTKDEYERHNSYTCEATHKTSTSPIVKSFNRNEC